European Patent Specification EP 3 710 579 B1, published April 12, 2023. Title: TREATMENT. Applicant: QUEEN MARY UNIVERSITY OF LONDON. The sequence listing filed with the application follows.

SEQUENCE LISTING (31 sequences)

SEQ ID NO: 1 - RNA, 21 nt, Artificial Sequence
  Synthetic construct
aagucuacaaaggucaccugu

SEQ ID NO: 2 - RNA, 29 nt, Artificial Sequence
  Synthetic construct
aagucuacaaaggucaccuguccugucuc

SEQ ID NO: 3 - RNA, 21 nt, Artificial Sequence
  Synthetic construct
aaacaggugaccuuuguagac

SEQ ID NO: 4 - RNA, 27 nt, Artificial Sequence
  Synthetic construct
aaacaggugaccuguagacccugucuc

SEQ ID NO: 5 - protein, 943 aa, Homo sapiens [sequence omitted]

SEQ ID NO: 6 - DNA, 3310 bp, Homo sapiens
ggacgcatcgtagaaaggggtggtggcgcccgaccccgcgccccggcccgaagctctgagggcttcccggcccccactgcctgcggcatggcccggggctcggcgctcccgcggcggccgctgctgtgcatcccggccgtctgggcggccgccgcgcttctgctctcagtgtcccggacttcaggtgaagtggaggttctggatccgaacgaccctttaggaccccttgatgggcaggacggcccgattccaactctgaaaggttactttctgaattttctggagccagtaaacaatatcaccattgtccaaggccagacggcaattctgcactgcaaggtggcaggaaacccaccccctaacgtgcggtggctaaagaatgatgccccggtggtgcaggagccgcggcggatcatcatccggaagacagaatatggttcacgactgcgaatccaggacctggacacgacagacactggctactaccagtgcgtggccaccaacgggatgaagaccattaccgccactggcgtcctgtttgtgcggctgggtccaacgcacagcccaaatcataactttcaggatgattaccacgaggatgggttctgccagccttaccggggaattgcctgtgcacgcttcattggcaaccggaccatttatgtggactcgcttcagatgcagggggagattgaaaaccgaatcacagcggccttcaccatgatcggcacgtctacgcacctgtcggaccagtgctcacagttcgccatcccatccttctgccacttcgtgtttcctctgtgcgacgcgcgctcccgggcacccaagccgcgtgagctgtgccgcgacgagtgcgaggtgctggagagcgacctgtgccgccaggagtacaccatcgcccgctccaacccgctcatcctcatgcggcttcagctgcccaagtgtgaggcgctgcccatgcctgagagccccgacgctgccaactgcatgcgcattggcatcccagccgagaggctgggccgctaccatcagtgctataacggctcaggcatggattacagaggaacggcaagcaccaccaagtcaggccaccagtgccagccgtgggccctgcagcacccccacagccaccacctgtccagcacagacttccctgagcttggaggggggcacgcctactgccggaaccccggaggccagatggagggcccctggtgctttacgcagaataaaaacgtacgcatggaactgtgtgacgtaccctcgtgtagtccccgagacagcagcaagatggggattctgtacatcttggtccccagcatcgcaattccactggtcatcgcttgccttttcttcttggtttgcatgtgccggaataagcagaaggcatctgcgtccacaccgcagcggcgacagctgatggcctcgcccagccaagacatggaaatgcccctcattaaccagcacaaacaggccaaactcaaagagatcagcctgtctgcggtgaggttcatggaggagctgggagaggaccggtttgggaaagtctacaaaggtcacctgttcggccctgccccgggggagcagacccaggctgtggccatcaaaacgctgaaggacaaagcggaggggcccctgcgggaggagttccggcatgaggctatgctgcgagcacggctgcaacaccccaacgtcgtctgcctgctgggcgtggtgaccaaggaccagcccctgagcatgatcttcagctactgttcgcacggcgacctccacgaattcctggtcatgcgctcgccgcactcggacgtgggcagcaccgatgatgaccgcacggtgaagtccgccctggagccccccgacttcgtgcaccttgtggcacagatcgcggcggggatggagtacctatccagccaccacgtggttcacaaggacctggccacccgcaatgtgctagtgtacgacaagctgaacgtgaagatctcagacttgggcctcttccgagaggtgtatgccgccgattactacaagctgctggggaactcgctgctgcctatccgctggatggccccagaggccatcatgtacggcaagttctccatcgactcagacatctggtcctacggtgtggtcctgtgggaggtcttcagctacggcctgcagccctactgcgggtattccaaccaggatgtggtggagatgatccggaaccggcaggtgctgccttgccccgatgactgtcccgcctgggtgtatgccctcatgatcgagtgctggaacgagttccccagccggcggccccgcttcaaggacatccacagccggctccgagcctggggcaacctttccaactacaacagctcggcgcagacctcgggggccagcaacaccacgcagaccagctccctgagcaccagcccagtgagcaatgtgagcaacgcccgctacgtggggcccaagcagaaggccccgcccttcccacagccccagttcatccccatgaagggccagatcagacccatggtgcccccgccgcagctctacatccccgtcaacggctaccagccggtgccggcctatggggcctacctgcccaacttctacccggtgcagatcccaatgcagatggccccgcagcaggtgcctcctcagatggtccccaagcccagctcacaccacagtggcagtggctccaccagcacaggctacgtcaccacggccccctccaacacatccatggcagacagggcagccctgctctcagagggcgctgatgacacacagaacgccccagaagatggggcccagagcaccgtgcaggaagcagaggaggaggaggaaggctctgtcccagagactgagctgctgggggactgtgacactctgcaggtggacgaggcccaagtccagctggaagcttgagtggcaccagggcccagggttcggggatagaagccccgccgagaccccacagggacctcagtcacctttgagaagacaccatactcagcaatcacaagagcccgccggccagtgggcttgtttgcagactgggtgaggtggagccctgctcctctctgtcctctgacacagctgccctgcctaggagcacccaagccaggcagggggtctggcagcacggcgtcctggggagcaggacacatggtcatccccagggctgtatacattgattctggtggtagactggtagtgagcagcaaatgcctttcaagaaaataggtggcagcttcactccatgtcatatatggagtgaatatttcaaaacgttgggaataagggcctgcaaaaggca

SEQ ID NO: 7 - protein, 944 aa, Mus musculus
MARGWVRPSRVPLCARAVWTAAALLLWTPWTAGEVEDSEAIDTLGQPDGPDSPLPTLKGYFLNFLEPVNNITIVQGQTAILHCKVAGNPPPNVRWLKNDAPVVQEPRRVIIRKTEYGSRLRIQDLDTTDTGYYQCVATNGLKTITATGVLYVRLGPTHSPNHNFQDDDQEDGFCQPYRGIACARFIGNRTIYVDSLQMQGEIENRITAAFTMIGTSTQLSDQCSQFAIPSFCHFVFPLCDARSRAPKPRELCRDECEVLENDLCRQEYTIARSNPLILMRLQLPKCEALPMPESPDAANCMRIGIPAERLGRYHQCYNGSGADYRGMASTTKSGHQCQPWALQHPHSHRLSSTEFPELGGGHAYCRNPGGQVEGPWCFTQNKNVRVELCDVPPCSPRDGSKMGILYILVPSIAIPLVIACLFFLVCMCRNKQKASASTPQRRQLMASPSQDMEMPLISQHKQAKLKEISLSTVRFMEELGEDRFGKVYKGHLFGPAPGEPTQAVAIKTLKDKAEGPLREEFRQEAMLRARLQHPNIVCLLGVVTKDQPLSMIFSYCSHGDLHEFLVMRSPHSDVGSTDDDRTVKSALEPPDFVHVVAQIAAGMEFLSSHHVVHKDLATRNVLVYDKLNVRISDLGLFREVYSADYYKLMGNSLLPIRWMSPEAVMYGKFSIDSDIWSYGVVLWEVFSYGLQPYCGYSNQDVVEMIRSRQVLPCPDDCPAWVYALMIECWNEFPSRRPRFKDIHSRLRSWGNLSNYNSSAQTSGASNTTQTSSLSTSPVSNVSNARYMAPKQKAQPFPQPQFIPMKGQIRPLVPPAQLYIPVNGYQPVPAYGAYLPNFYPVQIPMQMAPQQVPPQMVPKPSSHHSGSGSTSTGYVTTAPSNTSVADRAALLSEGTEDAQNIAEDVAQSPVQEAEEEEEGSVPETELLGDNDTLQVTEAAHVQLEA

SEQ ID NO: 8 - DNA, 2835 bp, Mus musculus
atggctcggggctgggtgcggccgagccgtgtgcctctgtgcgcccgggccgtctggacggctgcggcgctcctgctctggacaccctggacggcaggtgaagtggaagattcggaggcaatcgacaccttgggacaacctgatggaccggacagcccacttcccactctgaaaggctactttctgaattttctggagccagtcaacaatatcaccattgttcagggccagacggcaatcctgcactgcaaggtggcgggaaacccacctcccaatgtgcggtggctgaagaatgatgccccggttgtgcaagagccacgaagggtcgtcatccggaagacagaatacggctcccggctgcggatccaagacctggacacaacagacacaggctactaccagtgtgtggctaccaacgggctgaagaccatcactgccactggggttctatatgtgcggctcggtccgacgcacagcccgaaccacaattttcaggatgacgatcaggaagatggcttctgccagccgtaccgagggatcgcttgtgcgcgcttcattgggaaccggactatttatgtggactccctccagatgcagggggagattgaaaaccgaatcacagctgccttcaccatgatcggcacctccacgcaactgtcagaccagtgttcacagtttgccatcccatccttctgccacttcgtcttccctctgtgcgacgcatgctcccgggcgcccaagcctcgcgaactgtgccgggatgaatgtgaggtgctggagaacgacctgtgccgccaggagtacaccatcgcccgctccaacccgctcatcctcatgcggctccagctgcccaagtgcgaagcgctgcccatgcccgagagcccggatgctgcgaactgcatgcgcatcgggatccccgcggagaggctgggtcgctaccaccagtgctacaacggctccggcgccgattacagggggatggccagtaccaccaagtcaggccaccagtgtcagccttgggctctgcagcacccccacagccatcgcctatccagcacggaattccctgagctgggaggaggccatgcctactgccggaaccccgggggccagatggaaggcccgtggtgctttacgcagaataaaaacgtacgcgtggaactgtgtgacgtacccccgtgtagtccccgatatggcagcaagatggggattctgtacatcctggtccccagcattgctatccccctggtcatcgcttgcctgttcttcctcgtctgcatgtgccgcaacaaacagaaggcttcggcctccaccccacagcgccggcagctgatggcctctcccagccaggacatggagatgccactcatcagccagcacaaacaggccaaactcaaagagatcagcttgtccacagtgaggttcatggaggagctcggggaggaccggtttggcaaggtctacaaaggccacctgttcgggcctgccccaggagaaccaacccaggccgtggccatcaagacgctgaaagacaaggctgaggggcccctgcgggaggagttccggcaagaggcgatgctccgggcccgactgcagcaccccaacatcgtctgtctcctaggcgtcgtgaccaaggaccaacccttgagcatgatcttcagctactgttcccatggcgaccttcatgaattcctggtcatgcgctcgccgcactccgatgtgggcagcaccgatgacgaccgcacagtgaagtcagccctggagcccccggacttcgtgcacgtggtggcgcagatcgctgcggggatggagttcctgtccagccaccacgtgtgccataaggacctggccacacgcaatgtgctggtgtacgacaagctgaacgtgaggatctcagacttgggcctcttccgtgaggtatactccgcagattactacaaactcatgggcaattcactgctgcccatccgctggatgtcccccgaggccgtcatgtatggaaagttctccatcgactctgacatctggtcctacggtgtggtcctctgggaggtctttagctacggcctgcagccctactgtgggtactccaaccaggacgtggtggagatgatccggagccggcaggtgctgccctgcccggatgactgccccgcctgggtctatgccctcatgattgaatgctggaatgagttcccaagccggaggccccgctttaaggacatccacagccggctccggtcctggggcaacctatccaactataatagttccgcgcagacctcaggagccagcaacaccacacagaccagctccctgagcaccagccccgtaagcaatgtgagcaatgcccgctatatggcccccaagcagaaggcccagcccttcccacagcctcagttcatccccatgaagggtcagatcagacccttggtgccccccgcacagctgtacatcccggtgaacggctatcagccggtaccggcatacggggcctacctgcccaacttctacccagtccagatccccatgcagatggccccacagcaggtgccccctcagatggtccccaagccgagctcacaccacagtggcagcggctccaccagcactggctacgtcaccacggcgccctccaatacatctgtggcggacagggcggccctactctctgagggcaccgaggatgtacagaacatcgcggaagacgtggcccagagccctgtgcaggaagcagaggaggaggaggaggggtctgtccctgagactgaactcctgggagacaatgacacgctccaggtgaccgaggcggctcatgtccagcttgaagcctga

SEQ ID NO: 9 - protein, 25 aa, Artificial Sequence
  Synthetic construct
SSSTTTTTTTTLLLLLLLLLLLLLL

SEQ ID NO: 10 - protein, 406 aa, Homo sapiens
MARGSALPRRPLLCIPAVWAAAALLLSVSRTSGEVEVLDPNDPLGPLDGQDGPIPTLKGYFLNFLEPVNNITIVQGQTAILHCKVAGNPPPNVRWLKNDAPVVQEPRRIIIRKTEYGSRLRIQDLDTTDTGYYQCVATNGMKTITATGVLFVRLGPTHSPNHNFQDDYHEDGFCQPYRGIACARFIGNRTIYVDSLQMQGEIENRITAAFTMIGTSTHLSDQCSQFAIPSFCHFVFPLCDARSRAPKPRELCRDECEVLESDLCRQEYTIARSNPLILMRLQLPKCEALPMPESPDAANCMRIGIPAERLGRYHQCYNGSGMDYRGTASTTKSGHQCQPWALQHPHSHHLSSTDFPELGGGHAYCRNPGGQMEGPWCFTQNKNVRMELCDVPSCSPRDSSKMGILY

SEQ ID NO: 11 - DNA, 1218 bp, Homo sapiens
atggcccggggctcggcgctcccgcggcggccgctgctgtgcatcccggccgtctgggcggccgccgcgcttctgctctcagtgtcccggacttcaggtgaagtggaggttctggatccgaacgaccctttaggaccccttgatgggcaggacggcccgattccaactctgaaaggttactttctgaattttctggagccagtaaacaatatcaccattgtccaaggccagacggcaattctgcactgcaaggtggcaggaaacccaccccctaacgtgcggtggctaaagaatgatgccccggtggtgcaggagccgcggcggatcatcatccggaagacagaatatggttcacgactgcgaatccaggacctggacacgacagacactggctactaccagtgcgtggccaccaacgggatgaagaccattaccgccactggcgtcctgtttgtgcggctgggtccaacgcacagcccaaatcataactttcaggatgattaccacgaggatgggttctgccagccttaccggggaattgcctgtgcacgcttcattggcaaccggaccatttatgtggactcgcttcagatgcagggggagattgaaaaccgaatcacagcggccttcaccatgatcggcacgtctacgcacctgtcggaccagtgctcacagttcgccatcccatccttctgccacttcgtgtttcctctgtgcgacgcgcgctcccgggcacccaagccgcgtgagctgtgccgcgacgagtgcgaggtgctggagagcgacctgtgccgccaggagtacaccatcgcccgctccaacccgctcatcctcatgcggcttcagctgcccaagtgtgaggcgctgcccatgcctgagagccccgacgctgccaactgcatgcgcattggcatcccagccgagaggctgggccgctaccatcagtgctataacggctcaggcatggattacagaggaacggcaagcaccaccaagtcaggccaccagtgccagccgtgggccctgcagcacccccacagccaccacctgtccagcacagacttccctgagcttggaggggggcacgcctactgccggaaccccggaggccagatggagggcccctggtgctttacgcagaataaaaacgtacgcatggaactgtgtgacgtaccctcgtgtagtccccgagacagcagcaagatggggattctgtac

SEQ ID NO: 12 - protein, 126 aa, Homo sapiens
CQPYRGIACARFIGNRTIYVDSLQMQGEIENRITAAFTMIGTSTHLSDQCSQFAIPSFCHFVFPLCDARSRAPKPRELCRDECEVLESDLCRQEYTIARSNPLILMRLQLPKCEALPMPESPDAAN

SEQ ID NO: 13 - DNA, 379 bp, Homo sapiens
ctgccagccttaccggggaattgcctgtgcacgcttcattggcaaccggaccatttatgtggactcgcttcagatgcagggggagattgaaaaccgaatcacagcggccttcaccatgatcggcacgtctacgcacctgtcggaccagtgctcacagttcgccatcccatccttctgccacttcgtgtttcctctgtgcgacgcgcgctcccgggcacccaagccgcgtgagctgtgccgcgacgagtgcgaggtgctggagagcgacctgtgccgccaggagtacaccatcgcccgctccaacccgctcatcctcatgcggcttcagctgcccaagtgtgaggcgctgcccatgcctgagagccccgacgctgccaac

SEQ ID NO: 14 - DNA, 75 bp, Artificial Sequence
  Synthetic construct
agcagcagcaccaccaccaccaccaccaccaccctgctgctgctgctgctgctgctgctgctgctgctgctgctg

SEQ ID NO: 15 - RNA, 29 nt, Artificial Sequence
  Synthetic construct
gguucacgacugcgaauccaggaccugga

SEQ ID NO: 16 - RNA, 29 nt, Artificial Sequence
  Synthetic construct
aagaccauuaccgccacuggcguccuguu

SEQ ID NO: 17 - RNA, 29 nt, Artificial Sequence
  Synthetic construct
auggauuacagaggaacggcaagcaccac

SEQ ID NO: 18 - RNA, 29 nt, Artificial Sequence
  Synthetic construct
aagcagaaggcaucugcguccacaccgca

SEQ ID NO: 19 - RNA, 29 nt, Artificial Sequence
  Synthetic construct
ccuugagcaugaucuucagcuacuguucc

SEQ ID NO: 20 - protein, 5 aa, Artificial Sequence
  Synthetic construct
KDDDD

SEQ ID NO: 21 - DNA, 15 bp, Artificial Sequence
  Synthetic construct
aaagatgatgatgat

SEQ ID NO: 22 - DNA, 156 bp, Artificial Sequence
  Synthetic construct
agcagcagcaccaccaccaccaccaccaccaccctgctgctgctgctgctgctgctgctgctgctgctgctgctgaaagatgatgatgatgaacaaaaactcatctcagaagaggatctgaatatgcataccggtcatcatcaccatcaccattga

SEQ ID NO: 23 - protein, 7 aa, Artificial Sequence
  Tobacco etch virus protease cleavage tag
GQFYLNE

SEQ ID NO: 24 - DNA, 21 bp, Artificial Sequence
  Tobacco etch virus protease cleavage tag
ggccagttttatctgaacgaa

SEQ ID NO: 25 - DNA, 162 bp, Artificial Sequence
  Tobacco etch virus protease cleavage tag
agcagcagcaccaccaccaccaccaccaccaccctgctgctgctgctgctgctgctgctgctgctgctgctgctgggccagttttatctgaacgaagaacaaaaactcatctcagaagaggatctgaatatgcataccggtcatcatcaccatcaccattga

SEQ ID NO: 26 - protein, 431 aa, Artificial Sequence
  Synthetic construct
MARGSALPRRPLLCIPAVWAAAALLLSVSRTSGEVEVLDPNDPLGPLDGQDGPIPTLKGYFLNFLEPVNNITIVQGQTAILHCKVAGNPPPNVRWLKNDAPVVQEPRRIIIRKTEYGSRLRIQDLDTTDTGYYQCVATNGMKTITATGVLFVRLGPTHSPNHNFQDDYHEDGFCQPYRGIACARFIGNRTIYVDSLQMQGEIENRITAAFTMIGTSTHLSDQCSQFAIPSFCHFVFPLCDARSRAPKPRELCRDECEVLESDLCRQEYTIARSNPLILMRLQLPKCEALPMPESPDAANCMRIGIPAERLGRYHQCYNGSGMDYRGTASTTKSGHQCQPWALQHPHSHHLSSTDFPELGGGHAYCRNPGGQMEGPWCFTQNKNVRMELCDVPSCSPRDSSKMGILYSSSTTTTTTTTLLLLLLLLLLLLLL

SEQ ID NO: 27 - DNA, 1374 bp, Artificial Sequence
  Synthetic construct
atggcccggggctcggcgctcccgcggcggccgctgctgtgcatcccggccgtctgggcggccgccgcgcttctgctctcagtgtcccggacttcaggtgaagtggaggttctggatccgaacgaccctttaggaccccttgatgggcaggacggcccgattccaactctgaaaggttactttctgaattttctggagccagtaaacaatatcaccattgtccaaggccagacggcaattctgcactgcaaggtggcaggaaacccaccccctaacgtgcggtggctaaagaatgatgccccggtggtgcaggagccgcggcggatcatcatccggaagacagaatatggttcacgactgcgaatccaggacctggacacgacagacactggctactaccagtgcgtggccaccaacgggatgaagaccattaccgccactggcgtcctgtttgtgcggctgggtccaacgcacagcccaaatcataactttcaggatgattaccacgaggatgggttctgccagccttaccggggaattgcctgtgcacgcttcattggcaaccggaccatttatgtggactcgcttcagatgcagggggagattgaaaaccgaatcacagcggccttcaccatgatcggcacgtctacgcacctgtcggaccagtgctcacagttcgccatcccatccttctgccacttcgtgtttcctctgtgcgacgcgcgctcccgggcacccaagccgcgtgagctgtgccgcgacgagtgcgaggtgctggagagcgacctgtgccgccaggagtacaccatcgcccgctccaacccgctcatcctcatgcggcttcagctgcccaagtgtgaggcgctgcccatgcctgagagccccgacgctgccaactgcatgcgcattggcatcccagccgagaggctgggccgctaccatcagtgctataacggctcaggcatggattacagaggaacggcaagcaccaccaagtcaggccaccagtgccagccgtgggccctgcagcacccccacagccaccacctgtccagcacagacttccctgagcttggaggggggcacgcctactgccggaaccccggaggccagatggagggcccctggtgctttacgcagaataaaaacgtacgcatggaactgtgtgacgtaccctcgtgtagtccccgagacagcagcaagatggggattctgtacagcagcagcaccaccaccaccaccaccaccaccctgctgctgctgctgctgctgctgctgctgctgctgctgctgaaagatgatgatgatgaacaaaaactcatctcagaagaggatctgaatatgcataccggtcatcatcaccatcaccattga

SEQ ID NO: 28 - protein, 457 aa, Artificial Sequence
  Synthetic construct
MARGSALPRRPLLCIPAVWAAAALLLSVSRTSGEVEVLDPNDPLGPLDGQDGPIPTLKGYFLNFLEPVNNITIVQGQTAILHCKVAGNPPPNVRWLKNDAPVVQEPRRIIIRKTEYGSRLRIQDLDTTDTGYYQCVATNGMKTITATGVLFVRLGPTHSPNHNFQDDYHEDGFCQPYRGIACARFIGNRTIYVDSLQMQGEIENRITAAFTMIGTSTHLSDQCSQFAIPSFCHFVFPLCDARSRAPKPRELCRDECEVLESDLCRQEYTIARSNPLILMRLQLPKCEALPMPESPDAANCMRIGIPAERLGRYHQCYNGSGMDYRGTASTTKSGHQCQPWALQHPHSHHLSSTDFPELGGGHAYCRNPGGQMEGPWCFTQNKNVRMELCDVPSCSPRDSSKMGILYSSSTTTTTTTTLLLLLLLLLLLLLLKDDDDEQKLISEEDLNMHTGHHHHHH

SEQ ID NO: 29 - DNA, 1374 bp, Artificial Sequence; identical to SEQ ID NO: 27
  Synthetic construct

SEQ ID NO: 30 - protein, 459 aa, Artificial Sequence
  Synthetic construct
MARGSALPRRPLLCIPAVWAAAALLLSVSRTSGEVEVLDPNDPLGPLDGQDGPIPTLKGYFLNFLEPVNNITIVQGQTAILHCKVAGNPPPNVRWLKNDAPVVQEPRRIIIRKTEYGSRLRIQDLDTTDTGYYQCVATNGMKTITATGVLFVRLGPTHSPNHNFQDDYHEDGFCQPYRGIACARFIGNRTIYVDSLQMQGEIENRITAAFTMIGTSTHLSDQCSQFAIPSFCHFVFPLCDARSRAPKPRELCRDECEVLESDLCRQEYTIARSNPLILMRLQLPKCEALPMPESPDAANCMRIGIPAERLGRYHQCYNGSGMDYRGTASTTKSGHQCQPWALQHPHSHHLSSTDFPELGGGHAYCRNPGGQMEGPWCFTQNKNVRMELCDVPSCSPRDSSKMGILYSSSTTTTTTTTLLLLLLLLLLLLLLGQFYLNEEQKLISEEDLNMHTGHHHHHH

SEQ ID NO: 31 - DNA, 1380 bp, Artificial Sequence
  Synthetic construct
atggcccggggctcggcgctcccgcggcggccgctgctgtgcatcccggccgtctgggcggccgccgcgcttctgctctcagtgtcccggacttcaggtgaagtggaggttctggatccgaacgaccctttaggaccccttgatgggcaggacggcccgattccaactctgaaaggttactttctgaattttctggagccagtaaacaatatcaccattgtccaaggccagacggcaattctgcactgcaaggtggcaggaaacccaccccctaacgtgcggtggctaaagaatgatgccccggtggtgcaggagccgcggcggatcatcatccggaagacagaatatggttcacgactgcgaatccaggacctggacacgacagacactggctactaccagtgcgtggccaccaacgggatgaagaccattaccgccactggcgtcctgtttgtgcggctgggtccaacgcacagcccaaatcataactttcaggatgattaccacgaggatgggttctgccagccttaccggggaattgcctgtgcacgcttcattggcaaccggaccatttatgtggactcgcttcagatgcagggggagattgaaaaccgaatcacagcggccttcaccatgatcggcacgtctacgcacctgtcggaccagtgctcacagttcgccatcccatccttctgccacttcgtgtttcctctgtgcgacgcgcgctcccgggcacccaagccgcgtgagctgtgccgcgacgagtgcgaggtgctggagagcgacctgtgccgccaggagtacaccatcgcccgctccaacccgctcatcctcatgcggcttcagctgcccaagtgtgaggcgctgcccatgcctgagagccccgacgctgccaactgcatgcgcattggcatcccagccgagaggctgggccgctaccatcagtgctataacggctcaggcatggattacagaggaacggcaagcaccaccaagtcaggccaccagtgccagccgtgggccctgcagcacccccacagccaccacctgtccagcacagacttccctgagcttggaggggggcacgcctactgccggaaccccggaggccagatggagggcccctggtgctttacgcagaataaaaacgtacgcatggaactgtgtgacgtaccctcgtgtagtccccgagacagcagcaagatggggattctgtacagcagcagcaccaccaccaccaccaccaccaccctgctgctgctgctgctgctgctgctgctgctgctgctgctgggccagttttatctgaacgaagaacaaaaactcatctcagaagaggatctgaatatgcataccggtcatcatcaccatcaccattga